European Patent Application EP 4 644 530 A1, published November 5, 2025. Title: LEUCONOSTOC AND USE THEREOF. Applicant: Bloomage Biotechnology Corporation Limited. Application CN. The sequence listing filed with the application follows.

SEQUENCE LISTING (1 sequence)

SEQ ID NO: 1 - RNA, 1485 nt, synthetic construct
  source 1..1485: mol_type = other RNA
ctcaggatgaacgctggcggcgtgcctaatacatgcaagtcgaacgcacagcgaaaggtgcttgcacctttcaagtgagtggcgaacgggtgagtaacacgtggacaacctgcctcaaggctggggataacatttggaaacagatgctaataccgaataaaacttagtgtcgcatgacacaaagttaaaaggcgcttcggcgtcacctagagatggatccgcggtgcattagttagttggtggggtaaaggcctaccaagacaatgatgcatagccgagttgagagactgatcggccacattgggactgagacacggcccaaactcctacgggaggctgcagtagggaatcttccacaatgggcgaaagcctgatggagcaacgccgcgtgtgtgatgaaggctttcgggtcgtaaagcactgttgtatgggaagaacagctagaataggaaatgattttagtttgacggtaccataccagaaagggacggctaaatacgtgccagcagccgcggtaatacgtatgtcccgagcgttatccggatttattgggcgtaaagcgagcgcagacggtttattaagtctgatgtgaaagcccggagctcaactccggaatggcattggaaactggttaacttgagtgcagtagaggtaagtggaactccatgtgtagcggtggaatgcgtagatatatggaagaacaccagtggcgaaggcggcttactggactgcaactgacgttgaggctcgaaagtgtgggtagcaaacaggattagataccctggtagtccacaccgtaaacgatgaacactaggtgttaggaggtttccgcctcttagtgccgaagctaacgcattaagtgttccgcctggggagtacgaccgcaaggttgaaactcaaaggaattgacggggacccgcacaagcggtggagcatgtggtttaattcgaagcaacgcgaagaaccttaccaggtcttgacatcctttgaagcttttagagatagaagtgttctcttcggagacaaagtgacaggtggtgcatggtcgtcgtcagctcgtgtcgtgagatgttgggttaagtcccgcaacgagcgcaacccttattgttagttgccagcattcagatgggcactctagcgagactgccggtgacaaaccggaggaaggcggggacgacgtcagatcatcatgccccttatgacctgggctacacacgtgctacaatggcgtatacaacgagttgccaacccgcgagggtgagctaatctcttaaagtacgtctcagttcggattgtagtctgcaactcgactacatgaagtcggaatcgctagtaatcgcggatcagcacgccgcggtgaatacgttcccgggtcttgtacacaccgcccgtcacaccatgggagtttgtaatgcccaaagccggtggcctaaccttttaggaaggagccgtctaaggcaggacagatgactggggtgaagtcgt